European Patent Specification EP 2 701 737 B1, published March 27, 2024. Title: TOLEROGENIC SYNTHETIC NANOCARRIERS FOR ALLERGY THERAPY. Applicant: Selecta Biosciences, Inc. Fraser, Christopher Kishimoto, Takashi Maldonado, Roberto. The sequence listing filed with the application follows.

SEQUENCE LISTING (516 sequences)

SEQ ID NO: 1 - protein, 20 aa, Artificial Sequence
  Arachis hypogaea 2S protein 1 epitope
AHASARQQWELQGDRRCQSQ

SEQ ID NO: 2 - protein, 20 aa, Artificial Sequence
  Arachis hypogaea 2S protein 1 epitope
AKLTILVALALFLLAAHASA

SEQ ID NO: 3 - protein, 19 aa, Artificial Sequence
  Arachis hypogaea 2S protein 1 epitope
ALQQIMENQSDRLQGRQQE

SEQ ID NO: 4 - protein, 20 aa, Artificial Sequence
  Arachis hypogaea 2S protein 1 epitope
ANLRPCEQHLMQKIQRDEDS

SEQ ID NO: 5 - protein, 20 aa, Artificial Sequence
  Arachis hypogaea 2S protein 1 epitope
CNELNEFENNQRCMCEALQQ

SEQ ID NO: 6 - protein, 16 aa, Artificial Sequence
  Homo sapiens 5-hydroxytryptamine receptor 2C (5-HT-2C) (Serotonin receptor 2C) (5-HT2C) (5-HTR2C) (5HT-1C) epitope
PRGTMQAINNERKASK

SEQ ID NO: 7 - protein, 12 aa, Artificial Sequence
  Bos taurus Allergen Bos d 2 precursor epitope
DQGTCLLLTEVA

SEQ ID NO: 8 - protein, 14 aa, Artificial Sequence
  Bos taurus Allergen Bos d 2 precursor epitope
ELEKYQQLNSERGV

SEQ ID NO: 9 - protein, 13 aa, Artificial Sequence
  Bos taurus Allergen Bos d 2 precursor epitope
GERITKMTEGLAK

SEQ ID NO: 10 - protein, 14 aa, Artificial Sequence
  Bos taurus Allergen Bos d 2 precursor epitope
PGEWRIIYAAADNK

SEQ ID NO: 11 - protein, 8 aa, Artificial Sequence
  Bos taurus Allergen Bos d 2 precursor epitope
RIECINDC

SEQ ID NO: 12 - protein, 12 aa, Artificial Sequence
  Bos taurus Allergen Bos d 2 precursor epitope
VAKRQEGYVYVL

SEQ ID NO: 13 - protein, 10 aa, Artificial Sequence
  Bos taurus Allergen Bos d 2 precursor epitope
VSENMLVTYV

SEQ ID NO: 14 - protein, 16 aa, Artificial Sequence
  Bos taurus Allergen Bos d 2 precursor epitope
ELEKYQQLNSERGVPN

SEQ ID NO: 15 - protein, 13 aa, Artificial Sequence
  Cryptomeria japonica Allergen Cry j 2 epitope
DIFASKNFHLQKN

SEQ ID NO: 16 - protein, 13 aa, Artificial Sequence
  Cryptomeria japonica Allergen Cry j 2 epitope
GIIAAYQNPASWK

SEQ ID NO: 17 - protein, 12 aa, Artificial Sequence
  Cryptomeria japonica Allergen Cry j 2 epitope
KLTSGKIASCLN

SEQ ID NO: 18 - protein, 12 aa, Artificial Sequence
  Cryptomeria japonica Allergen Cry j 2 epitope
QFAKLTGFTLMG

SEQ ID NO: 19 - protein, 8 aa, Artificial Sequence
  Aspergillus fumigatus allergen I/a; Asp f I/a epitope
INQQLNPK

SEQ ID NO: 20 - protein, 15 aa, Artificial Sequence
  Aspergillus fumigatus allergen I/a; Asp f I/a epitope
INQQLNPKTNKWEDK

SEQ ID NO: 21 - protein, 11 aa, Artificial Sequence
  Aspergillus fumigatus allergen I/a; Asp f I/a epitope
LNPKTNKWEDK

SEQ ID NO: 22 - protein, 7 aa, Artificial Sequence
  Aspergillus fumigatus allergen I/a; Asp f I/a epitope
TNKWEDK

SEQ ID NO: 23 - protein, 12 aa, Artificial Sequence
  Aspergillus fumigatus allergen I/a; Asp f I/a epitope
LNPKTNKWEDKR

SEQ ID NO: 24 - protein, 15 aa, Artificial Sequence
  Dermatophagoides farinae Allergen Mag epitope
PRLSWHQYTKRDSRE

SEQ ID NO: 25 - protein, 15 aa, Artificial Sequence
  Dermatophagoides farinae Allergen Mag epitope
TVDLISPVTKRASLK

SEQ ID NO: 26 - protein, 18 aa, Artificial Sequence
  Bos taurus Alpha-S1-casein precursor epitope
AWYYVPLGTQYTDAPSFS

SEQ ID NO: 27 - protein, 18 aa, Artificial Sequence
  Bos taurus Alpha-S1-casein precursor epitope
DAYPSGAWYYVPLGTQYT

SEQ ID NO: 28 - protein, 18 aa, Artificial Sequence
  Bos taurus Alpha-S1-casein precursor epitope
DIGSESTEDQAMEDIKQM

SEQ ID NO: 29 - protein, 6 aa, Artificial Sequence
  Bos taurus Alpha-S1-casein precursor epitope
EDIKQM

SEQ ID NO: 30 - protein, 12 aa, Artificial Sequence
  Bos taurus Alpha-S1-casein precursor epitope
EPMIGVNQELAY

SEQ ID NO: 31 - protein, 18 aa, Artificial Sequence
  Bos taurus Alpha-S1-casein precursor epitope
EPMIGVNQELAYFYPELF

SEQ ID NO: 32 - protein, 17 aa, Artificial Sequence
  Arachis hypogaea Ara h 2.01 allergen epitope
ELNEFENNQRCMCEALQ

SEQ ID NO: 33 - protein, 16 aa, Artificial Sequence
  Arachis hypogaea Ara h 2.01 allergen epitope
SQLERANLRPCEQHLM

SEQ ID NO: 34 - protein, 15 aa, Artificial Sequence
  Cryptomeria japonica Cry j 1 precursor epitope
GATRDRPLWIIFSGN

SEQ ID NO: 35 - protein, 20 aa, Artificial Sequence
  Cryptomeria japonica Cry j 1 precursor epitope
IFSGNMNIKLKMPMYIAGYK

SEQ ID NO: 36 - protein, 20 aa, Artificial Sequence
  Cryptomeria japonica Cry j 1 precursor epitope
KMPMYIAGYKTFDGRGAQVY

SEQ ID NO: 37 - protein, 20 aa, Artificial Sequence
  Cryptomeria japonica Cry j 1 precursor epitope
LGHDDAYSDDKSMKVTVAFN

SEQ ID NO: 38 - protein, 19 aa, Artificial Sequence
  Cryptomeria japonica Cry j 1 precursor epitope
SGKYEGGNIYTKKEAFNVE

SEQ ID NO: 39 - protein, 11 aa, Artificial Sequence
  Cochliobolus lunatus Cytochrome c epitope
ENPKKYIPGTK

SEQ ID NO: 40 - protein, 11 aa, Artificial Sequence
  Cochliobolus lunatus Cytochrome c epitope
GLFGRKTGSVA

SEQ ID NO: 41 - protein, 9 aa, Artificial Sequence
  Cochliobolus lunatus Cytochrome c epitope
KIGPELHGL

SEQ ID NO: 42 - protein, 12 aa, Artificial Sequence
  Cochliobolus lunatus Cytochrome c epitope
LKAGEGNKIGPE

SEQ ID NO: 43 - protein, 11 aa, Artificial Sequence
  Cochliobolus lunatus Cytochrome c epitope
LKKPKDRNDLI

SEQ ID NO: 44 - protein, 18 aa, Artificial Sequence
  Dermatophagoides farinae Der f 2 allergen epitope
GLEIDVPGIDTNACHFVK

SEQ ID NO: 45 - protein, 20 aa, Artificial Sequence
  Dermatophagoides farinae Der f 2 allergen epitope
PGIDTNACHFVKCPLVKGQQ

SEQ ID NO: 46 - protein, 19 aa, Artificial Sequence
  Dermatophagoides pteronyssinus Der p 1 allergen epitope
RFGISNYCQIYPPNANKIR

SEQ ID NO: 47 - protein, 15 aa, Artificial Sequence
  Dermatophagoides pteronyssinus Der p 1 allergen epitope
AVNIVGYSNAQGVDY

SEQ ID NO: 48 - protein, 20 aa, Artificial Sequence
  Chironomus thummi globin Ctt 3-1 epitope
FAGKDLESIKGTAPFETHAN

SEQ ID NO: 49 - protein, 11 aa, Artificial Sequence
  Chironomus thummi globin Ctt 3-1 epitope
GTAPFETHANR

SEQ ID NO: 50 - protein, 21 aa, Artificial Sequence
  Chironomus thummi globin Ctt 3-1 epitope
KGTAPFETHANRIVGFFSKII

SEQ ID NO: 51 - protein, 21 aa, Artificial Sequence
  Chironomus thummi thummi Globin CTT-III epitope
AHTDFAGAEAAWGATLDTFFG

SEQ ID NO: 52 - protein, 20 aa, Artificial Sequence
  Chironomus thummi thummi Globin CTT-III epitope
FAGKDLESIKGTAPFEIHAN

SEQ ID NO: 53 - protein, 21 aa, Artificial Sequence
  Chironomus thummi thummi Globin CTT-III epitope
VNTFVASHKPRGVTHDQLNNF

SEQ ID NO: 54 - protein, 8 aa, Artificial Sequence
  Chironomus thummi thummi Globin CTT-III precursor epitope
ADPSIMAK

SEQ ID NO: 55 - protein, 21 aa, Artificial Sequence
  Chironomus thummi thummi Globin CTT-III precursor epitope
ADPSIMAKFTQFAGKDLESIK

SEQ ID NO: 56 - protein, 5 aa, Artificial Sequence
  Chironomus thummi thummi Globin CTT-III precursor epitope
AEAAW

SEQ ID NO: 57 - protein, 20 aa, Artificial Sequence
  Chironomus thummi thummi Globin CTT-III precursor epitope
AEAAWGATLDTFFGMIFSKM

SEQ ID NO: 58 - protein, 8 aa, Artificial Sequence
  Chironomus thummi thummi Globin CTT-III precursor epitope
AGFVSYMK

SEQ ID NO: 59 - protein, 15 aa, Artificial Sequence
  Phaseolus vulgaris Glycine-rich cell wall structural protein 1.8 precursor epitope
GGYGDGGAHGGGYGG

SEQ ID NO: 60 - protein, 15 aa, Artificial Sequence
  Phleum pratense Group V allergen Phl p 5 epitope
ATPEAKYDAYVATLS

SEQ ID NO: 61 - protein, 15 aa, Artificial Sequence
  Phleum pratense Group V allergen Phl p 5 epitope
FTVFEAAFNNAIKAG

SEQ ID NO: 62 - protein, 15 aa, Artificial Sequence
  Phleum pratense Group V allergen Phl p 5 epitope
KYDAYVATLSEALRI

SEQ ID NO: 63 - protein, 15 aa, Artificial Sequence
  Phleum pratense Group V allergen Phl p 5 epitope
PANDKFTVFEAAFNN

SEQ ID NO: 64 - protein, 15 aa, Artificial Sequence
  Phleum pratense Group V allergen Phl p 5 epitope
PKGGAESSSKAALTS

SEQ ID NO: 65 - protein, 16 aa, Artificial Sequence
  Homo sapiens KIAA1224 protein epitope
DLESYLQLNCERGTWR

SEQ ID NO: 66 - protein, 15 aa, Artificial Sequence
  Lepidoglyphus destructor Lep D 2 precursor epitope
KGEALDFNYGMTIPA

SEQ ID NO: 67 - protein, 12 aa, Artificial Sequence
  Corylus avellana lipid transfer protein precursor epitope
AGLPGKCGVNIP

SEQ ID NO: 68 - protein, 12 aa, Artificial Sequence
  Corylus avellana lipid transfer protein precursor epitope
AKGIAGLNPNLA

SEQ ID NO: 69 - protein, 12 aa, Artificial Sequence
  Corylus avellana lipid transfer protein precursor epitope
CGVNIPYKISPS

SEQ ID NO: 70 - protein, 12 aa, Artificial Sequence
  Corylus avellana lipid transfer protein precursor epitope
CKGVRAVNDASR

SEQ ID NO: 71 - protein, 12 aa, Artificial Sequence
  Corylus avellana lipid transfer protein precursor epitope
CVLYLKNGGVLP

SEQ ID NO: 72 - protein, 16 aa, Artificial Sequence
  Homo sapiens Lipocalin 1 (tear prealbumin) epitope
KPVRGVKLVGRDPKNN

SEQ ID NO: 73 - protein, 15 aa, Artificial Sequence
  Dermatophagoides farinae Mag3 epitope
EFNTEFTIHADKNNL

SEQ ID NO: 74 - protein, 15 aa, Artificial Sequence
  Dermatophagoides farinae Mag3 epitope
FTIHADKNNLKMHMD

SEQ ID NO: 75 - protein, 15 aa, Artificial Sequence
  Dermatophagoides farinae Mag3 epitope
KMHMDFPNVFQADLT

SEQ ID NO: 76 - protein, 13 aa, Artificial Sequence
  Apium graveolens Major allergen Api g 1 epitope
ALFKALEAYLIAN

SEQ ID NO: 77 - protein, 12 aa, Artificial Sequence
  Apium graveolens Major allergen Api g 1 epitope
DAVVPEENIKYA

SEQ ID NO: 78 - protein, 12 aa, Artificial Sequence
  Apium graveolens Major allergen Api g 1 epitope
DILLGFIESIEN

SEQ ID NO: 79 - protein, 12 aa, Artificial Sequence
  Apium graveolens Major allergen Api g 1 epitope
GGSICKTTAIFH

SEQ ID NO: 80 - protein, 12 aa, Artificial Sequence
  Apium graveolens Major allergen Api g 1 epitope
GVQTHVLELTSS

SEQ ID NO: 81 - protein, 15 aa, Artificial Sequence
  Aspergillus fumigatus Major allergen Asp f 2 precursor epitope
FGNRPTMEAVGAYDV

SEQ ID NO: 82 - protein, 15 aa, Artificial Sequence
  Aspergillus fumigatus Major allergen Asp f 2 precursor epitope
MEAVGAYDVIVNGDK

SEQ ID NO: 83 - protein, 16 aa, Artificial Sequence
  Canis lupus familiaris Major allergen Can f 1 precursor epitope
ALEDFREFSRAKGLNQ

SEQ ID NO: 84 - protein, 16 aa, Artificial Sequence
  Canis lupus familiaris Major allergen Can f 1 precursor epitope
DQEVPEKPDSVTPMIL

SEQ ID NO: 85 - protein, 12 aa, Artificial Sequence
  Corylus avellana major allergen Cor a 1.0401 epitope
AGKEKAAGLFKA

SEQ ID NO: 86 - protein, 12 aa, Artificial Sequence
  Corylus avellana major allergen Cor a 1.0401 epitope
AGLFKAVEAYLL

SEQ ID NO: 87 - protein, 12 aa, Artificial Sequence
  Corylus avellana major allergen Cor a 1.0401 epitope
APQHFTSAENLE

SEQ ID NO: 88 - protein, 12 aa, Artificial Sequence
  Corylus avellana major allergen Cor a 1.0401 epitope
ARLFKSFVLDAD

SEQ ID NO: 89 - protein, 12 aa, Artificial Sequence
  Corylus avellana major allergen Cor a 1.0401 epitope
EIDHANFKYCYS

SEQ ID NO: 90 - protein, 13 aa, Artificial Sequence
  Daucus carota Major allergen Dau c 1 epitope
ALFKAIEAYLIAN

SEQ ID NO: 91 - protein, 16 aa, Artificial Sequence
  Equus caballus Major allergen Equ c 1 precursor epitope
DGYNVFRISEFENDEH

SEQ ID NO: 92 - protein, 16 aa, Artificial Sequence
  Equus caballus Major allergen Equ c 1 precursor epitope
DKDRPFQLFEFYAREP

SEQ ID NO: 93 - protein, 16 aa, Artificial Sequence
  Equus caballus Major allergen Equ c 1 precursor epitope
DLTKIDRCFQLRGNGV

SEQ ID NO: 94 - protein, 16 aa, Artificial Sequence
  Equus caballus Major allergen Equ c 1 precursor epitope
DRPFQLFEFYAREPDV

SEQ ID NO: 95 - protein, 16 aa, Artificial Sequence
  Equus caballus Major allergen Equ c 1 precursor epitope
DVSPEIKEEFVKIVQK

SEQ ID NO: 96 - protein, 17 aa, Artificial Sequence
  Felis catus major allergen I epitope
ENARILKNCVDAKMTEE

SEQ ID NO: 97 - protein, 17 aa, Artificial Sequence
  Felis catus major allergen I epitope
RDVDLFLTGTPDEYVEQ

SEQ ID NO: 98 - protein, 17 aa, Artificial Sequence
  Felis catus major allergen I epitope
TGTPDEYVEQVAQYKAL

SEQ ID NO: 99 - protein, 17 aa, Artificial Sequence
  Felis catus Major allergen I polypeptide chain 1 precursor epitope
DVDLFLTGTPDEYVEQV

SEQ ID NO: 100 - protein, 17 aa, Artificial Sequence
  Felis catus Major allergen I polypeptide chain 1 precursor epitope
EICPAVKRDVDLFLTGT

SEQ ID NO: 101 - protein, 16 aa, Artificial Sequence
  Felis catus Major allergen I polypeptide chain 1 precursor epitope
EQVAQYKALPVVLENA

SEQ ID NO: 102 - protein, 17 aa, Artificial Sequence
  Felis catus Major allergen I polypeptide chain 1 precursor epitope
KALPVVLENARILKNCV

SEQ ID NO: 103 - protein, 17 aa, Artificial Sequence
  Felis catus Major allergen I polypeptide chain 1 precursor epitope
LFLTGTPDEYVEQVAQY

SEQ ID NO: 104 - protein, 16 aa, Artificial Sequence
  Felis catus major allergen I, polypeptide chain 1 epitope
KENALSLLDKIYTSPL

SEQ ID NO: 105 - protein, 16 aa, Artificial Sequence
  Felis catus major allergen I, polypeptide chain 1 epitope
KMTEEDKENALSLLDK

SEQ ID NO: 106 - protein, 15 aa, Artificial Sequence
  Malus x domestica Major allergen Mal d 1 epitope
GLFKLIESYLKDHPD

SEQ ID NO: 107 - protein, 15 aa, Artificial Sequence
  Prunus avium Major allergen Pru av 1 epitope
NLFKLIETYLKGHPD

SEQ ID NO: 108 - protein, 20 aa, Artificial Sequence
  Hevea brasiliensis Major latex allergen Hev b 5 epitope
AAPAEGEKPAEEEKPITEAA

SEQ ID NO: 109 - protein, 20 aa, Artificial Sequence
  Hevea brasiliensis Major latex allergen Hev b 5 epitope
AEEEKPITEAAETATTEVPV

SEQ ID NO: 110 - protein, 20 aa, Artificial Sequence
  Hevea brasiliensis Major latex allergen Hev b 5 epitope
APAEPEAPAPETEKAEEVEK

SEQ ID NO: 111 - protein, 20 aa, Artificial Sequence
  Hevea brasiliensis Major latex allergen Hev b 5 epitope
APEADQTTPEEKPAEPEPVA

SEQ ID NO: 112 - protein, 20 aa, Artificial Sequence
  Hevea brasiliensis Major latex allergen Hev b 5 epitope
ASEQETADATPEKEEPTAAP

SEQ ID NO: 113 - protein, 11 aa, Artificial Sequence
  Dermatophagoides pteronyssinus Major mite fecal allergen Der p 1 epitope
YAYVAREQSCR

SEQ ID NO: 114 - protein, 19 aa, Artificial Sequence
  Dermatophagoides pteronyssinus Major mite fecal allergen Der p 1 epitope
ALAQTHTAIAVIIGIKDLD

SEQ ID NO: 115 - protein, 35 aa, Artificial Sequence
  Olea europaea Major pollen allergen epitope
EDIPQPPVSQFHIQGQVYCDTCRAGFITELSEFIP

SEQ ID NO: 116 - protein, 31 aa, Artificial Sequence
  Olea europaea Major pollen allergen epitope
GASLRLQCKDKENGDVTFTEVGYTRAEGLYS

SEQ ID NO: 117 - protein, 34 aa, Artificial Sequence
  Olea europaea Major pollen allergen epitope
GTTRTVNPLGFFKKEALPKCAQVYNKLGMYPPNM

SEQ ID NO: 118 - protein, 53 aa, Artificial Sequence
  Olea europaea Major pollen allergen epitope
LVERDHKNEFCEITLISSGRKDCNEIPTEGWAKPSLKFKLNTVNGTTRTVNPL

SEQ ID NO: 119 - protein, 33 aa, Artificial Sequence
  Olea europaea Major pollen allergen epitope
MLVERDHKNEFCEITLISSGRKDCNEIPTEGWA

SEQ ID NO: 120 - protein, 12 aa, Artificial Sequence
  Artemisia vulgaris Major pollen allergen Art v 1 precursor epitope
AGGSPSPPADGG

SEQ ID NO: 121 - protein, 12 aa, Artificial Sequence
  Artemisia vulgaris Major pollen allergen Art v 1 precursor epitope
AGSKLCEKTSKT

SEQ ID NO: 122 - protein, 12 aa, Artificial Sequence
  Artemisia vulgaris Major pollen allergen Art v 1 precursor epitope
CDKKCIEWEKAQ

SEQ ID NO: 123 - protein, 12 aa, Artificial Sequence
  Artemisia vulgaris Major pollen allergen Art v 1 precursor epitope
DGGSPPPPADGG

SEQ ID NO: 124 - protein, 12 aa, Artificial Sequence
  Artemisia vulgaris Major pollen allergen Art v 1 precursor epitope
EKTSKTYSGKCD

SEQ ID NO: 125 - protein, 12 aa, Artificial Sequence
  Betula pendula Major pollen allergen Bet v 1-A epitope
AARLFKAFILDG

SEQ ID NO: 126 - protein, 15 aa, Artificial Sequence
  Betula pendula Major pollen allergen Bet v 1-A epitope
AARLFKAFILDGDNL

SEQ ID NO: 127 - protein, 12 aa, Artificial Sequence
  Betula pendula Major pollen allergen Bet v 1-A epitope
AEQVKASKEMGE

SEQ ID NO: 128 - protein, 21 aa, Artificial Sequence
  Betula pendula Major pollen allergen Bet v 1-A epitope
AFILDGDNLFPKVAPQAISSV

SEQ ID NO: 129 - protein, 12 aa, Artificial Sequence
  Betula pendula Major pollen allergen Bet v 1-A epitope
AISSVENIEGNG

SEQ ID NO: 130 - protein, 15 aa, Artificial Sequence
  Betula pendula Major pollen allergen Bet v 1-A epitope
ETLLRAVESYLLAHS

SEQ ID NO: 131 - protein, 16 aa, Artificial Sequence
  Betula pendula Major pollen allergen Bet v 1-F/I epitope
GETLLRAVESYLLAHS

SEQ ID NO: 132 - protein, 20 aa, Artificial Sequence
  Chamaecyparis obtusa Major pollen allergen Cha o 1 precursor epitope
ANNNYDPWSIYAIGGSSNPT

SEQ ID NO: 133 - protein, 20 aa, Artificial Sequence
  Chamaecyparis obtusa Major pollen allergen Cha o 1 precursor epitope
ASTGVTISNNHFFNHHKVML

SEQ ID NO: 134 - protein, 20 aa, Artificial Sequence
  Chamaecyparis obtusa Major pollen allergen Cha o 1 precursor epitope
CANWVWRSTQDSFNNGAYFV

SEQ ID NO: 135 - protein, 20 aa, Artificial Sequence
  Chamaecyparis obtusa Major pollen allergen Cha o 1 precursor epitope
DAITMRNVTDVWIDHNSLSD

SEQ ID NO: 136 - protein, 20 aa, Artificial Sequence
  Chamaecyparis obtusa Major pollen allergen Cha o 1 precursor epitope
DANWDQNRMKLADCAVGFGS

SEQ ID NO: 137 - protein, 20 aa, Artificial Sequence
  Cynodon dactylon Major pollen allergen Cyn d 1 epitope
AIGDKPGPNITATYGNKWLE

SEQ ID NO: 138 - protein, 20 aa, Artificial Sequence
  Cynodon dactylon Major pollen allergen Cyn d 1 epitope
CYEIKCKEPVECSGEPVLVK

SEQ ID NO: 139 - protein, 20 aa, Artificial Sequence
  Cynodon dactylon Major pollen allergen Cyn d 1 epitope
DHGGACGYKDVDKPPFDGMT

SEQ ID NO: 140 - protein, 20 aa, Artificial Sequence
  Cynodon dactylon Major pollen allergen Cyn d 1 epitope
EGGAHLVQDDVIPANWKPDT

SEQ ID NO: 141 - protein, 20 aa, Artificial Sequence
  Cynodon dactylon Major pollen allergen Cyn d 1 epitope
FKDGLGCGACYEIKCKEPVE

SEQ ID NO: 142 - protein, 15 aa, Artificial Sequence
  Phleum pratense Major pollen allergen Phl p 4 precursor epitope
FAEYKSDYVYQPFPK

SEQ ID NO: 143 - protein, 15 aa, Artificial Sequence
  Phleum pratense Major pollen allergen Phl p 4 precursor epitope
MLLRKYGIAAENVID

SEQ ID NO: 144 - protein, 15 aa, Artificial Sequence
  Phleum pratense Major pollen allergen Phl p 4 precursor epitope
NSFKPFAEYKSDYVY

SEQ ID NO: 145 - protein, 20 aa, Artificial Sequence
  Rattus norvegicus Major urinary protein precursor epitope
ASNKREKIEENGSMRVFMQH

SEQ ID NO: 146 - protein, 20 aa, Artificial Sequence
  Rattus norvegicus Major urinary protein precursor epitope
DIKEKFAKLCEAHGITRDNI

SEQ ID NO: 147 - protein, 20 aa, Artificial Sequence
  Rattus norvegicus Major urinary protein precursor epitope
EEASSTRGNLDVAKLNGDWF

SEQ ID NO: 148 - protein, 20 aa, Artificial Sequence
  Rattus norvegicus Major urinary protein precursor epitope
EENGSMRVFMQHIDVLENSL

SEQ ID NO: 149 - protein, 20 aa, Artificial Sequence
  Rattus norvegicus Major urinary protein precursor epitope
ENSLGFKFRIKENGECRELY

SEQ ID NO: 150 - protein, 21 aa, Artificial Sequence
  Dermatophagoides farinae Mite group 2 allergen Der f 2 precursor epitope
DIKYTWNVPKIAPKSENVVVT

SEQ ID NO: 151 - protein, 17 aa, Artificial Sequence
  Dermatophagoides farinae Mite group 2 allergen Der f 2 precursor epitope
DNGVLACAIATHGKIRD

SEQ ID NO: 152 - protein, 21 aa, Artificial Sequence
  Dermatophagoides farinae Mite group 2 allergen Der f 2 precursor epitope
EALFDANQNTKTAKIEIKASL

SEQ ID NO: 153 - protein, 45 aa, Artificial Sequence
  Dermatophagoides farinae Mite group 2 allergen Der f 2 precursor epitope
QYDIKYTWNVPKIAPKSENVVVTVKLIGDNGVLACAIATHGKIRD

SEQ ID NO: 154 - protein, 19 aa, Artificial Sequence
  Dermatophagoides farinae Mite group 2 allergen Der f 2 precursor epitope
TKTAKIEIKASLDGLEIDV

SEQ ID NO: 155 - protein, 14 aa, Artificial Sequence
  Dermatophagoides pteronyssinus Mite group 2 allergen Der p 2 epitope
ASIDGLGVDVPGID

SEQ ID NO: 156 - protein, 15 aa, Artificial Sequence
  Dermatophagoides pteronyssinus Mite group 2 allergen Der p 2 epitope
FEAVQNTKTAKIEIK

SEQ ID NO: 157 - protein, 17 aa, Artificial Sequence
  Dermatophagoides pteronyssinus Mite group 2 allergen Der p 2 epitope
RGKPPQLEAVFEAVQNT

SEQ ID NO: 158 - protein, 15 aa, Artificial Sequence
  Dermatophagoides pteronyssinus Mite group 2 allergen Der p 2 precursor epitope
CHGSEPCIIHRGKPF

SEQ ID NO: 159 - protein, 27 aa, Artificial Sequence
  Dermatophagoides pteronyssinus Mite group 2 allergen Der p 2 precursor epitope
CPLVKGQQYDIKYTWNVPKIAPKSENV

SEQ ID NO: 160 - protein, 26 aa, Artificial Sequence
  Dermatophagoides pteronyssinus Mite group 2 allergen Der p 2 precursor epitope
DIKYTWNVPKIAPKSENVVVTVKVMG

SEQ ID NO: 161 - protein, 15 aa, Artificial Sequence
  Dermatophagoides pteronyssinus Mite group 2 allergen Der p 2 precursor epitope
DQVDVKDCANHEIKK

SEQ ID NO: 162 - protein, 20 aa, Artificial Sequence
  Dermatophagoides pteronyssinus Mite group 2 allergen Der p 2 precursor epitope
DQVDVKDCANHEIKKVLVPG

SEQ ID NO: 163 - protein, 15 aa, Artificial Sequence
  Lepidoglyphus destructor Mite group 2 allergen Lep d 2 precursor epitope
DHGVMACGTVHGQVE

SEQ ID NO: 164 - protein, 15 aa, Artificial Sequence
  Lepidoglyphus destructor Mite group 2 allergen Lep d 2 precursor epitope
GCKFIKCPVKKGEAL

SEQ ID NO: 165 - protein, 15 aa, Artificial Sequence
  Lepidoglyphus destructor Mite group 2 allergen Lep d 2 precursor epitope
GEKMTLEAKFAANQD

SEQ ID NO: 166 - protein, 15 aa, Artificial Sequence
  Lepidoglyphus destructor Mite group 2 allergen Lep d 2 precursor epitope
GEVTELDITGCSGDT

SEQ ID NO: 167 - protein, 15 aa, Artificial Sequence
  Lepidoglyphus destructor Mite group 2 allergen Lep d 2 precursor epitope
GKMTFKDCGHGEVTE

SEQ ID NO: 168 - protein, 16 aa, Artificial Sequence
  Homo sapiens Neurofilament heavy polypeptide (NF-H) (Neurofilament triplet H protein) (200 kDa neurofilament protein) epitope
YQEAIQQLDAELRNTK

SEQ ID NO: 169 - protein, 10 aa, Artificial Sequence
  Prunus persica Non-specific lipid-transfer protein 1 epitope
AAALPGKCGV

SEQ ID NO: 170 - protein, 10 aa, Artificial Sequence
  Prunus persica Non-specific lipid-transfer protein 1 epitope
ACCNGIRNVN

SEQ ID NO: 171 - protein, 10 aa, Artificial Sequence
  Prunus persica Non-specific lipid-transfer protein 1 epitope
APCIPYVRGG

SEQ ID NO: 172 - protein, 10 aa, Artificial Sequence
  Prunus persica Non-specific lipid-transfer protein 1 epitope
IRNVNNLART

SEQ ID NO: 173 - protein, 11 aa, Artificial Sequence
  Prunus persica Non-specific lipid-transfer protein 1 epitope
ISASTNCATVK

SEQ ID NO: 174 - protein, 10 aa, Artificial Sequence
  Prunus persica Non-specific lipid-transfer protein 1 epitope
NLARTTPDRQ

SEQ ID NO: 175 - protein, 10 aa, Artificial Sequence
  Gallus gallus Ovalbumin epitope
CFDVFKELKV

SEQ ID NO: 176 - protein, 10 aa, Artificial Sequence
  Gallus gallus Ovalbumin epitope
GSIGAASMEF

SEQ ID NO: 177 - protein, 18 aa, Artificial Sequence
  Gallus gallus Ovalbumin epitope
IGLFRVASMASEKMKILE

SEQ ID NO: 178 - protein, 18 aa, Artificial Sequence
  Gallus gallus Ovalbumin epitope
IKHIATNAVLFFGRCVSP

SEQ ID NO: 179 - protein, 13 aa, Artificial Sequence
  Gallus gallus Ovalbumin epitope
IMSALAMVYLGAK

SEQ ID NO: 180 - protein, 14 aa, Artificial Sequence
  Gallus gallus Ovomucoid precursor epitope
AEVDCSRFPNATDK

SEQ ID NO: 181 - protein, 14 aa, Artificial Sequence
  Gallus gallus Ovomucoid precursor epitope
ATDKEGKDVLVCNK

SEQ ID NO: 182 - protein, 17 aa, Artificial Sequence
  Gallus gallus Ovomucoid precursor epitope
AVVESNGTLTLSHFGKC

SEQ ID NO: 183 - protein, 16 aa, Artificial Sequence
  Gallus gallus Ovomucoid precursor epitope
CLLCAYSIEFGTNISK

SEQ ID NO: 184 - protein, 20 aa, Artificial Sequence
  Gallus gallus Ovomucoid precursor epitope
DNECLLCAHKVEQGASVDKR

SEQ ID NO: 185 - protein, 16 aa, Artificial Sequence
  Musa acuminata pectate lyase epitope
GHSDELTSDKSMQVTI

SEQ ID NO: 186 - protein, 16 aa, Artificial Sequence
  Zinnia violacea Pectate lyase precursor epitope
GHSDSYTQDKNMQVTI

SEQ ID NO: 187 - protein, 21 aa, Artificial Sequence
  Dermatophagoides farinae Peptidase 1 precursor (Major mite fecal allergen Der f 1) (Allergen Der f I) epitope
DGRTIIQHDNGYQPNYHAVNI

SEQ ID NO: 188 - protein, 19 aa, Artificial Sequence
  Dermatophagoides farinae Peptidase 1 precursor (Major mite fecal allergen Der f 1) (Allergen Der f I) epitope
DLRSLRTVTPIRMQGGCGS

SEQ ID NO: 189 - protein, 19 aa, Artificial Sequence
  Dermatophagoides farinae Peptidase 1 precursor (Major mite fecal allergen Der f 1) (Allergen Der f I) epitope
GCGSCWAFSGVAATESAYL

SEQ ID NO: 190 - protein, 21 aa, Artificial Sequence
  Dermatophagoides farinae Peptidase 1 precursor (Major mite fecal allergen Der f 1) (Allergen Der f I) epitope
IREALTQTHTAIAVIIGIKDL

SEQ ID NO: 191 - protein, 19 aa, Artificial Sequence
  Dermatophagoides farinae Peptidase 1 precursor (Major mite fecal allergen Der f 1) (Allergen Der f I) epitope
IRMQGGCGSCWAFSGVAAT

SEQ ID NO: 192 - protein, 19 aa, Artificial Sequence
  Euroglyphus maynei Peptidase 1 precursor (Mite group 1 allergen Eur m 1) (Allergen Eur m I) epitope
FRHYDGRTIMQHDNGYQPN

SEQ ID NO: 193 - protein, 19 aa, Artificial Sequence
  Euroglyphus maynei Peptidase 1 precursor (Mite group 1 allergen Eur m 1) (Allergen Eur m I) epitope
GRTIMQHDNGYQPNYHAVN

SEQ ID NO: 194 - protein, 19 aa, Artificial Sequence
  Euroglyphus maynei Peptidase 1 precursor (Mite group 1 allergen Eur m 1) (Allergen Eur m I) epitope
HAVNIVGYGNTQGVDYWIV

SEQ ID NO: 195 - protein, 19 aa, Artificial Sequence
  Euroglyphus maynei Peptidase 1 precursor (Mite group 1 allergen Eur m 1) (Allergen Eur m I) epitope
NKIRQALTQTHTAVAVIIG

SEQ ID NO: 196 - protein, 19 aa, Artificial Sequence
  Euroglyphus maynei Peptidase 1 precursor (Mite group 1 allergen Eur m 1) (Allergen Eur m I) epitope
PYVAREQSCHRPNAQRYGL

SEQ ID NO: 197 - protein, 15 aa, Artificial Sequence
  Phleum pratense Phl p 3 allergen epitope
AVQVTFTVQKGSDPK

SEQ ID NO: 198 - protein, 15 aa, Artificial Sequence
  Phleum pratense Phl p 3 allergen epitope
EEWEPLTKKGNVWEV

SEQ ID NO: 199 - protein, 15 aa, Artificial Sequence
  Phleum pratense Phl p 3 allergen epitope
FTVQKGSDPKKLVLD

SEQ ID NO: 200 - protein, 15 aa, Artificial Sequence
  Phleum pratense Phl p 3 allergen epitope
FTVQKGSDPKKLVLN

SEQ ID NO: 201 - protein, 15 aa, Artificial Sequence
  Phleum pratense Phl p 3 allergen epitope
GSDPKKLVLDIKYTR

SEQ ID NO: 202 - protein, 15 aa, Artificial Sequence
  Apis mellifera Phospholipase A2 precursor epitope
CDCDDKFYDCLKNSA

SEQ ID NO: 203 - protein, 12 aa, Artificial Sequence
  Apis mellifera Phospholipase A2 precursor epitope
CLHYTVDKSKPK

SEQ ID NO: 204 - protein, 15 aa, Artificial Sequence
  Apis mellifera Phospholipase A2 precursor epitope
CRTHDMCPDVMSAGE

SEQ ID NO: 205 - protein, 18 aa, Artificial Sequence
  Apis mellifera Phospholipase A2 precursor epitope
DTISSYFVGKMYFNLIDT

SEQ ID NO: 206 - protein, 18 aa, Artificial Sequence
  Apis mellifera Phospholipase A2 precursor epitope
ERTEGRCLHYTVDKSKPK

SEQ ID NO: 207 - protein, 16 aa, Artificial Sequence
  Spiroplasma citri plectrovirus spv1-r8a2b orf 14 transmembrane protein epitope
HVIEVQQINSERSWFF

SEQ ID NO: 208 - protein, 20 aa, Artificial Sequence
  Lolium perenne pollen allergen epitope
CGYKDVDKAPFNGMTGCGNT

SEQ ID NO: 209 - protein, 20 aa, Artificial Sequence
  Lolium perenne pollen allergen epitope
GAGPKDNGGACGYKDVDKAP

SEQ ID NO: 210 - protein, 20 aa, Artificial Sequence
  Lolium perenne pollen allergen epitope
SEVEDVIPEGWKADTSYSAK

SEQ ID NO: 211 - protein, 20 aa, Artificial Sequence
  Lolium perenne pollen allergen epitope
VEKGSNPNYLAILVKYVDGD

SEQ ID NO: 212 - protein, 20 aa, Artificial Sequence
  Lolium perenne pollen allergen epitope
YPDDTKPTFHVEKGSNPNYL

SEQ ID NO: 213 - protein, 16 aa, Artificial Sequence
  Ambrosia artemisiifolia Pollen allergen Amb a 1.1 precursor epitope
GAGDENIEDRGMLATV

SEQ ID NO: 214 - protein, 16 aa, Artificial Sequence
  Ambrosia artemisiifolia Pollen allergen Amb a 2 precursor epitope
GASDTHFQDLKMHVTL

SEQ ID NO: 215 - protein, 11 aa, Artificial Sequence
  Ambrosia artemisiifolia var. elatior Pollen allergen Amb a 3 epitope
EEAYHACDIKD

SEQ ID NO: 216 - protein, 15 aa, Artificial Sequence
  Ambrosia artemisiifolia var. elatior Pollen allergen Amb a 3 epitope
GKVYLVGGPELGGWK

SEQ ID NO: 217 - protein, 15 aa, Artificial Sequence
  Ambrosia artemisiifolia var. elatior Pollen allergen Amb a 3 epitope
LGGWKLQSDPRAYAL

SEQ ID NO: 218 - protein, 15 aa, Artificial Sequence
  Ambrosia artemisiifolia var. elatior Pollen allergen Amb a 3 epitope
PGGPDRFTLLTPGSH

SEQ ID NO: 219 - protein, 15 aa, Artificial Sequence
  Ambrosia artemisiifolia var. elatior Pollen allergen Amb a 5 epitope
AYCCSDPGRYCPWQV

SEQ ID NO: 220 - protein, 20 aa, Artificial Sequence
  Ambrosia artemisiifolia var. elatior Pollen allergen Amb a 5 epitope
CGEKRAYCCSDPGRYCPWQV

SEQ ID NO: 221 - protein, 17 aa, Artificial Sequence
  Ambrosia artemisiifolia var. elatior Pollen allergen Amb a 5 epitope
DPGRYCPWQVVCYESSE

SEQ ID NO: 222 - protein, 20 aa, Artificial Sequence
  Ambrosia artemisiifolia var. elatior Pollen allergen Amb a 5 epitope
DPGRYCPWQVVCYESSEICS

SEQ ID NO: 223 - protein, 15 aa, Artificial Sequence
  Ambrosia artemisiifolia var. elatior Pollen allergen Amb a 5 epitope
GNVCGEKRAYCCSDP

SEQ ID NO: 224 - protein, 15 aa, Artificial Sequence
  Ambrosia artemisiifolia var. elatior Pollen allergen Amb a 5 epitope
LVPCAWAGNVCGEKR

SEQ ID NO: 225 - protein, 20 aa, Artificial Sequence
  Ambrosia artemisiifolia var. elatior Pollen allergen Amb a 5 epitope
LVPCAWAGNVCGEKRAYCCS

SEQ ID NO: 226 - protein, 15 aa, Artificial Sequence
  Ambrosia artemisiifolia var. elatior Pollen allergen Amb a 5 epitope
VCYESSEICSKKCGK

SEQ ID NO: 227 - protein, 20 aa, Artificial Sequence
  Ambrosia trifida Pollen allergen Amb t 5 precursor epitope
CGKVGKYCCSPIGKYCVCYD

SEQ ID NO: 228 - protein, 20 aa, Artificial Sequence
  Ambrosia trifida Pollen allergen Amb t 5 precursor epitope
DDGLCYEGTNCGKVGKYCCS

SEQ ID NO: 229 - protein, 12 aa, Artificial Sequence
  Ambrosia trifida Pollen allergen Amb t 5 precursor epitope
GKYCVCYDSKAI

SEQ ID NO: 230 - protein, 14 aa, Artificial Sequence
  Ambrosia trifida Pollen allergen Amb t 5 precursor epitope
PIGKYCVCYDSKAI

SEQ ID NO: 231 - protein, 20 aa, Artificial Sequence
  Ambrosia trifida Pollen allergen Amb t 5 precursor epitope
PIGKYCVCYDSKAICNKNCT

SEQ ID NO: 232 - protein, 14 aa, Artificial Sequence
  Ambrosia trifida Pollen allergen Amb t 5 precursor epitope
VCYDSKAICNKNCT

SEQ ID NO: 233 - protein, 15 aa, Artificial Sequence
  Betula pendula pollen allergen Bet v 1 epitope
HEVKAEQVKATKEMG

SEQ ID NO: 234 - protein, 20 aa, Artificial Sequence
  Poa pratensis Pollen allergen KBG 60 precursor epitope
AANKYKTFVATFGAASNKAF

SEQ ID NO: 235 - protein, 20 aa, Artificial Sequence
  Poa pratensis Pollen allergen KBG 60 precursor epitope
AAPANDKFTVFEAAFNDAIK

SEQ ID NO: 236 - protein, 20 aa, Artificial Sequence
  Poa pratensis Pollen allergen KBG 60 precursor epitope
AAVDSSKAALTSKLDAAYKL

SEQ ID NO: 237 - protein, 20 aa, Artificial Sequence
  Poa pratensis Pollen allergen KBG 60 precursor epitope
AEEVKATPAGELQVIDKVDA

SEQ ID NO: 238 - protein, 20 aa, Artificial Sequence
  Poa pratensis Pollen allergen KBG 60 precursor epitope
AFKVAATAANAAPANDKFTV

SEQ ID NO: 239 - protein, 20 aa, Artificial Sequence
  Lolium perenne Pollen allergen Lol p 1 precursor epitope
AFGSMAKKGEEQNVRSAGEL

SEQ ID NO: 240 - protein, 20 aa, Artificial Sequence
  Lolium perenne Pollen allergen Lol p 1 precursor epitope
AGELELQFRRVKCKYPDDTK

SEQ ID NO: 241 - protein, 20 aa, Artificial Sequence
  Lolium perenne Pollen allergen Lol p 1 precursor epitope
AKSTWYGKPTGAGPKDNGGA

SEQ ID NO: 242 - protein, 20 aa, Artificial Sequence
  Lolium perenne Pollen allergen Lol p 1 precursor epitope
APYHFDLSGHAFGSMAKKGE

SEQ ID NO: 243 - protein, 12 aa, Artificial Sequence
  Lolium perenne Pollen allergen Lol p 1 precursor epitope
IAPYHFDLSGHA

SEQ ID NO: 244 - protein, 20 aa, Artificial Sequence
  Lolium perenne Pollen allergen Lol p VA precursor epitope
AALTKAITAMTQAQKAGKPA

SEQ ID NO: 245 - protein, 20 aa, Artificial Sequence
  Lolium perenne Pollen allergen Lol p VA precursor epitope
AANAAPTNDKFTVFESAFNK

SEQ ID NO: 246 - protein, 20 aa, Artificial Sequence
  Lolium perenne Pollen allergen Lol p VA precursor epitope
ADKFKIFEAAFSESSKGLLA

SEQ ID NO: 247 - protein, 20 aa, Artificial Sequence
  Lolium perenne Pollen allergen Lol p VA precursor epitope
AFSESSKGLLATSAAKAPGL

SEQ ID NO: 248 - protein, 20 aa, Artificial Sequence
  Lolium perenne Pollen allergen Lol p VA precursor epitope
AYAATVAAAPEVKYAVFEAA

SEQ ID NO: 249 - protein, 12 aa, Artificial Sequence
  Phleum pratense Pollen allergen Phl p 1 epitope
ACSGEPVVVHIT

SEQ ID NO: 250 - protein, 12 aa, Artificial Sequence
  Phleum pratense Pollen allergen Phl p 1 epitope
AEDVIPEGWKAD

SEQ ID NO: 251 - protein, 12 aa, Artificial Sequence
  Phleum pratense Pollen allergen Phl p 1 epitope
AGELELQFRRVK

SEQ ID NO: 252 - protein, 12 aa, Artificial Sequence
  Phleum pratense Pollen allergen Phl p 1 epitope
DKWIELKESWGA

SEQ ID NO: 253 - protein, 12 aa, Artificial Sequence
  Phleum pratense Pollen allergen Phl p 1 epitope
DKWLDAKSTWYG

SEQ ID NO: 254 - protein, 12 aa, Artificial Sequence
  Phleum pratense Pollen allergen Phl p 1 precursor epitope
FEIKCTKPEACS

SEQ ID NO: 255 - protein, 12 aa, Artificial Sequence
  Phleum pratense Pollen allergen Phl p 1 precursor epitope
YHFDLSGHAFGA

SEQ ID NO: 256 - protein, 15 aa, Artificial Sequence
  Phleum pratense Pollen allergen Phl p 1 precursor epitope
ELKESWGAIWRIDTP

SEQ ID NO: 257 - protein, 15 aa, Artificial Sequence
  Phleum pratense Pollen allergen Phl p 1 precursor epitope
EPIAPYHFDLSGHAF

SEQ ID NO: 258 - protein, 15 aa, Artificial Sequence
  Phleum pratense Pollen allergen Phl p 1 precursor epitope
FEIKCTKPEACSGEP

SEQ ID NO: 259 - protein, 15 aa, Artificial Sequence
  Phleum pratense Pollen allergen Phl p 1 precursor epitope
WGAIWRIDTPDKLTG

SEQ ID NO: 260 - protein, 15 aa, Artificial Sequence
  Phleum pratense Pollen allergen Phl p 11 epitope
RYANPIAFFRKEPLK

SEQ ID NO: 261 - protein, 15 aa, Artificial Sequence
  Phleum pratense Pollen allergen Phl p 2 epitope
EHGSDEWVAMTKGEG

SEQ ID NO: 262 - protein, 15 aa, Artificial Sequence
  Phleum pratense Pollen allergen Phl p 2 epitope
EWVAMTKGEGGVWTF

SEQ ID NO: 263 - protein, 15 aa, Artificial Sequence
  Phleum pratense Pollen allergen Phl p 2 epitope
GVWTFDSEEPLQGPF

SEQ ID NO: 264 - protein, 15 aa, Artificial Sequence
  Phleum pratense Pollen allergen Phl p 2 epitope
KNVFDDVVPEKYTIG

SEQ ID NO: 265 - protein, 15 aa, Artificial Sequence
  Phleum pratense Pollen allergen Phl p 2 epitope
LQGPFNFRFLTEKGM

SEQ ID NO: 266 - protein, 15 aa, Artificial Sequence
  Phleum pratense Pollen allergen Phl p 4 epitope
FKPFAEYKSDYVYEP

SEQ ID NO: 267 - protein, 15 aa, Artificial Sequence
  Phleum pratense Pollen allergen Phl p 4 epitope
FPKEVWEQIFSTWLL

SEQ ID NO: 268 - protein, 15 aa, Artificial Sequence
  Phleum pratense Pollen allergen Phl p 4 epitope
FVHLGHRDNIEDDLL

SEQ ID NO: 269 - protein, 15 aa, Artificial Sequence
  Phleum pratense Pollen allergen Phl p 4 epitope
GIVVAWKVRLLPVPP

SEQ ID NO: 270 - protein, 15 aa, Artificial Sequence
  Phleum pratense Pollen allergen Phl p 4 epitope
NRNNTFKPFAEYKSD

SEQ ID NO: 271 - protein, 12 aa, Artificial Sequence
  Phleum pratense Pollen allergen Phl p 5a epitope
EVKYTVFETALK

SEQ ID NO: 272 - protein, 19 aa, Artificial Sequence
  Phleum pratense Pollen allergen Phl p 5a epitope
NAGFKAALAGAGVQPADKY

SEQ ID NO: 273 - protein, 27 aa, Artificial Sequence
  Phleum pratense Pollen allergen Phl p 5b precursor epitope
AAGKATTEEQKLIEDINVGFKAAVAAA

SEQ ID NO: 274 - protein, 33 aa, Artificial Sequence
  Phleum pratense Pollen allergen Phl p 5b precursor epitope
AAGKATTEEQKLIEDINVGFKAAVAAAASVPAA

SEQ ID NO: 275 - protein, 19 aa, Artificial Sequence
  Phleum pratense Pollen allergen Phl p 5b precursor epitope
AAVAAAASVPAADKFKTFE

SEQ ID NO: 276 - protein, 27 aa, Artificial Sequence
  Phleum pratense Pollen allergen Phl p 5b precursor epitope
AKFDSFVASLTEALRVIAGALEVHAVK

SEQ ID NO: 277 - protein, 19 aa, Artificial Sequence
  Phleum pratense Pollen allergen Phl p 5b precursor epitope
AMSEVQKVSQPATGAATVA

SEQ ID NO: 278 - protein, 20 aa, Artificial Sequence
  Chamaecyparis obtusa Polygalacturonase epitope
ARWKNSKIWLQFAQLTDFNL

SEQ ID NO: 279 - protein, 20 aa, Artificial Sequence
  Chamaecyparis obtusa Polygalacturonase epitope
AVLLVPANKKFFVNNLVFRG

SEQ ID NO: 280 - protein, 20 aa, Artificial Sequence
  Chamaecyparis obtusa Polygalacturonase epitope
DGTIVAQPDPARWKNSKIWL

SEQ ID NO: 281 - protein, 20 aa, Artificial Sequence
  Chamaecyparis obtusa Polygalacturonase epitope
FFVNNLVFRGPCQPHLSFKV

SEQ ID NO: 282 - protein, 20 aa, Artificial Sequence
  Chamaecyparis obtusa Polygalacturonase epitope
FGECEGVKIQGLKIKAPRDS

SEQ ID NO: 283 - protein, 15 aa, Artificial Sequence
  Cryptomeria japonica Polygalacturonase precursor epitope
AAYQNPASWKNNRIW

SEQ ID NO: 284 - protein, 15 aa, Artificial Sequence
  Cryptomeria japonica Polygalacturonase precursor epitope
ACKKPSAMLLVPGNK

SEQ ID NO: 285 - protein, 15 aa, Artificial Sequence
  Cryptomeria japonica Polygalacturonase precursor epitope
AIKFDFSTGLIIQGL

SEQ ID NO: 286 - protein, 15 aa, Artificial Sequence
  Cryptomeria japonica Polygalacturonase precursor epitope
AINIFNVEKYGAVGD

SEQ ID NO: 287 - protein, 15 aa, Artificial Sequence
  Cryptomeria japonica Polygalacturonase precursor epitope
ANGYFSGHVIPACKN

SEQ ID NO: 288 - protein, 16 aa, Artificial Sequence
  Arabidopsis thaliana Probable pectate lyase 18 precursor epitope
GHSDTYSRDKNMQVTI

SEQ ID NO: 289 - protein, 15 aa, Artificial Sequence
  Phleum pratense Profilin-2/4 epitope
LGHDGTVWAQSADFP

SEQ ID NO: 290 - protein, 20 aa, Artificial Sequence
  Hevea brasiliensis Pro-hevein precursor epitope
DEYCSPDHNCQSNCKDSGEG

SEQ ID NO: 291 - protein, 20 aa, Artificial Sequence
  Hevea brasiliensis Pro-hevein precursor epitope
EQCGRQAGGKLCPNNLCCSQ

SEQ ID NO: 292 - protein, 43 aa, Artificial Sequence
  Hevea brasiliensis Pro-hevein precursor epitope
EQCGRQAGGKLCPNNLCCSQWGWCGSTDEYCSPDHNCQSNCKD

SEQ ID NO: 293 - protein, 20 aa, Artificial Sequence
  Hevea brasiliensis Pro-hevein precursor epitope
KLCPNNLCCSQWGWCGSTDE

SEQ ID NO: 294 - protein, 20 aa, Artificial Sequence
  Hevea brasiliensis Pro-hevein precursor epitope
NGGLDLDVNVFRQLDTDGKG

SEQ ID NO: 295 - protein, 10 aa, Artificial Sequence
  Prunus persica pru p 1 epitope
GKCGVSIPYK

SEQ ID NO: 296 - protein, 10 aa, Artificial Sequence
  Prunus persica pru p 1 epitope
ITCGQVSSSL

SEQ ID NO: 297 - protein, 10 aa, Artificial Sequence
  Prunus persica pru p 1 epitope
SIPYKISAST

SEQ ID NO: 298 - protein, 15 aa, Artificial Sequence
  Prunus persica pru p 1 epitope
DRQAACNCLKQLSAS

SEQ ID NO: 299 - protein, 15 aa, Artificial Sequence
  Prunus persica pru p 1 epitope
VNPNNAAALPGKCGV

SEQ ID NO: 300 - protein, 16 aa, Artificial Sequence
  Arabidopsis thaliana Putative pectate lyase 17 precursor epitope
GHNDNFVKDVKMKVTV

SEQ ID NO: 301 - protein, 16 aa, Artificial Sequence
  Homo sapiens RAD51-like 1 isoform 1 epitope
TRLILQYLDSERRQIL

SEQ ID NO: 302 - protein, 16 aa, Artificial Sequence
  Aspergillus fumigatus Ribonuclease mitogillin precursor epitope
DPGPARVIYTYPNKVF

SEQ ID NO: 303 - protein, 20 aa, Artificial Sequence
  Aspergillus fumigatus Ribonuclease mitogillin precursor epitope
ATWTCINQQLNPKTNKWEDK

SEQ ID NO: 304 - protein, 20 aa, Artificial Sequence
  Aspergillus fumigatus Ribonuclease mitogillin precursor epitope
HYLLEFPTFPDGHDYKFDSK

SEQ ID NO: 305 - protein, 20 aa, Artificial Sequence
  Aspergillus fumigatus Ribonuclease mitogillin precursor epitope
KFDSKKPKEDPGPARVIYTY

SEQ ID NO: 306 - protein, 20 aa, Artificial Sequence
  Aspergillus fumigatus Ribonuclease mitogillin precursor epitope
LIKGRTPIKFGKADCDRPPK

SEQ ID NO: 307 - protein, 20 aa, Artificial Sequence
  Aspergillus fumigatus Ribonuclease mitogillin precursor epitope
SYPHWFTNGYDGNGKLIKGR

SEQ ID NO: 308 - protein, 19 aa, Artificial Sequence
  Hevea brasiliensis Rubber elongation factor protein epitope
AEDEDNQQGQGEGLKYLGF

SEQ ID NO: 309 - protein, 19 aa, Artificial Sequence
  Hevea brasiliensis Rubber elongation factor protein epitope
FSNVYLFAKDKSGPLQPGV

SEQ ID NO: 310 - protein, 19 aa, Artificial Sequence
  Hevea brasiliensis Rubber elongation factor protein epitope
KFVDSTVVASVTIIDRSLP

SEQ ID NO: 311 - protein, 19 aa, Artificial Sequence
  Hevea brasiliensis Rubber elongation factor protein epitope
QPGVDIIEGPVKNVAVPLY

SEQ ID NO: 312 - protein, 19 aa, Artificial Sequence
  Hevea brasiliensis Rubber elongation factor protein epitope
RSLPPIVKDASIQVVSAIR

SEQ ID NO: 313 - protein, 17 aa, Artificial Sequence
  Bos taurus Serum albumin precursor epitope
DDSPDLPKLKPDPNTLC

SEQ ID NO: 314 - protein, 20 aa, Artificial Sequence
  Bos taurus Serum albumin precursor epitope
EKDAIPENLPPLTADFAEDK

SEQ ID NO: 315 - protein, 9 aa, Artificial Sequence
  Bos taurus Serum albumin precursor epitope
ESHAGCEKS

SEQ ID NO: 316 - protein, 10 aa, Artificial Sequence
  Bos taurus Serum albumin precursor epitope
HPEYAVSVLL

SEQ ID NO: 317 - protein, 9 aa, Artificial Sequence
  Bos taurus Serum albumin precursor epitope
LSLILNRLC

SEQ ID NO: 318 - protein, 12 aa, Artificial Sequence
  Hevea brasiliensis Small rubber particle protein epitope
DFVRAAGVYAVD

SEQ ID NO: 319 - protein, 12 aa, Artificial Sequence
  Hevea brasiliensis Small rubber particle protein epitope
KYLDFVRAAGVY

SEQ ID NO: 320 - protein, 12 aa, Artificial Sequence
  Hevea brasiliensis Small rubber particle protein epitope
NVVKTVVTPVYY

SEQ ID NO: 321 - protein, 12 aa, Artificial Sequence
  Hevea brasiliensis Small rubber particle protein epitope
PRIVLDVASSVF

SEQ ID NO: 322 - protein, 12 aa, Artificial Sequence
  Hevea brasiliensis Small rubber particle protein epitope
QGYRVSSYLPLL

SEQ ID NO: 323 - protein, 15 aa, Artificial Sequence
  Glycine max Stress-induced protein SAM22 epitope
ALFKAIEAYLLAHPD

SEQ ID NO: 324 - protein, 15 aa, Artificial Sequence
  Cryptomeria japonica Sugi basic protein precursor epitope
AFNVENGNATPQLTK

SEQ ID NO: 325 - protein, 15 aa, Artificial Sequence
  Cryptomeria japonica Sugi basic protein precursor epitope
ANNNYDPWTIYAIGG

SEQ ID NO: 326 - protein, 15 aa, Artificial Sequence
  Cryptomeria japonica Sugi basic protein precursor epitope
AYSDDKSMKVTVAFN

SEQ ID NO: 327 - protein, 15 aa, Artificial Sequence
  Cryptomeria japonica Sugi basic protein precursor epitope
CGQRMPRARYGLVHV

SEQ ID NO: 328 - protein, 15 aa, Artificial Sequence
  Cryptomeria japonica Sugi basic protein precursor epitope
CSNWVWQSTQDVFYN

SEQ ID NO: 329 - protein, 20 aa, Artificial Sequence
  Trichophyton rubrum Tri r 2 allergen epitope
ADFSNYGAVVDVYAPGKDIT

SEQ ID NO: 330 - protein, 20 aa, Artificial Sequence
  Trichophyton rubrum Tri r 2 allergen epitope
AKGVSLVAVKVLDCDGSGSN

SEQ ID NO: 331 - protein, 20 aa, Artificial Sequence
  Trichophyton rubrum Tri r 2 allergen epitope
ASNQAAKAISDAGIFMAVAA

SEQ ID NO: 332 - protein, 20 aa, Artificial Sequence
  Trichophyton rubrum Tri r 2 allergen epitope
DCNGHGTHVAGTVGGTKYGL

SEQ ID NO: 333 - protein, 20 aa, Artificial Sequence
  Trichophyton rubrum Tri r 2 allergen epitope
DPSAGKGVTAYIIDTGIDID

SEQ ID NO: 334 - protein, 12 aa, Artificial Sequence
  Vespula vulgaris Venom allergen 5 precursor epitope
ACKYGSLKPNCG

SEQ ID NO: 335 - protein, 12 aa, Artificial Sequence
  Vespula vulgaris Venom allergen 5 precursor epitope
CNYGPSGNFMNE

SEQ ID NO: 336 - protein, 12 aa, Artificial Sequence
  Vespula vulgaris Venom allergen 5 precursor epitope
DVAKYQVGQNVA

SEQ ID NO: 337 - protein, 12 aa, Artificial Sequence
  Vespula vulgaris Venom allergen 5 precursor epitope
EKWHKHYLVCNY

SEQ ID NO: 338 - protein, 12 aa, Artificial Sequence
  Vespula vulgaris Venom allergen 5 precursor epitope
ELAYVAQVWANQ

SEQ ID NO: 339 - protein, 15 aa, Artificial Sequence
  Corylus avellana 11S globulin-like protein epitope
AFQISREEARRLKYN

SEQ ID NO: 340 - protein, 12 aa, Artificial Sequence
  Carya illinoinensis 11S legumin protein epitope
EESQRQSQQGQR

SEQ ID NO: 341 - protein, 18 aa, Artificial Sequence
  Fagopyrum esculentum 13S globulin epitope
DAHQPTRRVRKGDVVALP

SEQ ID NO: 342 - protein, 12 aa, Artificial Sequence
  Fagopyrum esculentum 13S globulin seed storage protein 1 precursor (Legumin-like protein 1) epitope
FKQNVNRPSRAD

SEQ ID NO: 343 - protein, 12 aa, Artificial Sequence
  Fagopyrum esculentum 13S globulin seed storage protein 3 precursor (Legumin-like protein 3) (Allergen Fag e 1) epitope
DISTKEAFRLKN

SEQ ID NO: 344 - protein, 12 aa, Artificial Sequence
  Anacardium occidentale 2s albumin epitope
CQRQFEEQQRFR

SEQ ID NO: 345 - protein, 10 aa, Artificial Sequence
  Sesamum indicum 2S seed storage protein 1 epitope
HFRECCNEIR

SEQ ID NO: 346 - protein, 10 aa, Artificial Sequence
  Sesamum indicum 2S seed storage protein 1 precursor epitope
CMQWMRSMRG

SEQ ID NO: 347 - protein, 14 aa, Artificial Sequence
  Bertholletia excelsa 2S sulfur-rich seed storage protein precursor (Allergen Ber e 1) epitope
CRCEGLRMMMMRMQ

SEQ ID NO: 348 - protein, 21 aa, Artificial Sequence
  Cynodon dactylon acidic Cyn d 1 isoallergen isoform 1 precursor epitope
QDDVIPEDWKPDTVYKSKIQF

SEQ ID NO: 349 - protein, 50 aa, Artificial Sequence
  Cynodon dactylon acidic Cyn d 1 isoallergen isoform 3 precursor epitope
EEDKLRKAGELMLQFRRVKCEYPSDTKITFHVEKGSSPNYLALLVKYAAG

SEQ ID NO: 350 - protein, 7 aa, Artificial Sequence
  Bos taurus albumin epitope
PVESKVT

SEQ ID NO: 351 - protein, 13 aa, Artificial Sequence
  Juglans regia Albumin seed storage protein epitope
GLRGEEMEEMVQS

SEQ ID NO: 352 - protein, 18 aa, Artificial Sequence
  Cochliobolus lunatus alcohol dehydrogenase epitope
AVNGDWPLPTKLPLVGGH

SEQ ID NO: 353 - protein, 37 aa, Artificial Sequence
  Penicillium chrysogenum alkaline serine protease epitope
ANVVQRNAPSWGLSRISSKKSGATDYVYDSTAGEGIV

SEQ ID NO: 354 - protein, 10 aa, Artificial Sequence
  Arachis hypogaea allergen epitope
DDQCQRQLQR

SEQ ID NO: 355 - protein, 15 aa, Artificial Sequence
  Anacardium occidentale allergen Ana o 2 epitope
EESEDEKRRWGQRDN

SEQ ID NO: 356 - protein, 10 aa, Artificial Sequence
  Arachis hypogaea Allergen Ara h 1, clone P41B precursor epitope
AKSSPYQKKT

SEQ ID NO: 357 - protein, 15 aa, Artificial Sequence
  Arachis hypogaea allergen Arah3/Arah4 epitope
AGVALSRLVLRRNAL

SEQ ID NO: 358 - protein, 10 aa, Artificial Sequence
  Arachis hypogaea allergen Arah6 epitope
DRQMVQHFKR

SEQ ID NO: 359 - protein, 11 aa, Artificial Sequence
  Periplaneta americana Allergen Cr-PI epitope
IPKGKKGGQAY

SEQ ID NO: 360 - protein, 8 aa, Artificial Sequence
  Aspergillus fumigatus allergen I/a; Asp f I/a epitope
INQQLNPK

SEQ ID NO: 361 - protein, 10 aa, Artificial Sequence
  Arachis hypogaea Allergen II epitope
DRLQGRQQEQ

SEQ ID NO: 362 - protein, 15 aa, Artificial Sequence
  Lens culinaris allergen Len c 1.0101 epitope
AINASSDLNLIGFGI

SEQ ID NO: 363 - protein, 12 aa, Artificial Sequence
  Dermatophagoides farinae Allergen Mag epitope
DVELSLRSSDIA

SEQ ID NO: 364 - protein, 31 aa, Artificial Sequence
  Penicillium chrysogenum Allergen Pen n 18 epitope
AHIKKSKKGDKKFKGSVANMSLGGGSSRTLD

SEQ ID NO: 365 - protein, 14 aa, Artificial Sequence
  Sinapis alba Allergen Sin a 1 epitope
QGPHVISRIYQTAT

SEQ ID NO: 366 - protein, 12 aa, Artificial Sequence
  Ziziphus mauritiana allergen Ziz m 1 epitope
KTNYSSSIILEY

SEQ ID NO: 367 - protein, 37 aa, Artificial Sequence
  Fagopyrum tataricum allergenic protein epitope
DISTEEAYKLKNGRQEVEVFRPFQSRYEKEEEKERER

SEQ ID NO: 368 - protein, 30 aa, Artificial Sequence
  Bos taurus alpha S1 casein epitope
EDQAMEDIKQMEAESISSSEEIVPNSVEQK

SEQ ID NO: 369 - protein, 10 aa, Artificial Sequence
  Triticum aestivum Alpha/beta-gliadin A-II precursor epitope
QVSFQQPQQQ

SEQ ID NO: 370 - protein, 10 aa, Artificial Sequence
  Triticum aestivum Alpha/beta-gliadin A-V epitope
LALQTLPAMC

SEQ ID NO: 371 - protein, 20 aa, Artificial Sequence
  Bos taurus alpha2(I) collagen epitope
LPGLKGHNGLQGLPGLAGHH

SEQ ID NO: 372 - protein, 5 aa, Artificial Sequence
  Triticum aestivum Alpha-amylase inhibitor 0.28 precursor (CIII) (WMAI-1) epitope
AYPDV

SEQ ID NO: 373 - protein, 12 aa, Artificial Sequence
  Triticum aestivum Alpha-gliadin epitope
LGQGSFRPSQQN

SEQ ID NO: 374 - protein, 10 aa, Artificial Sequence
  Bos taurus Alpha-lactalbumin epitope
KDLKGYGGVS

SEQ ID NO: 375 - protein, 14 aa, Artificial Sequence
  Bos taurus Alpha-lactalbumin precursor epitope
KCEVFRELKDLKGY

SEQ ID NO: 376 - protein, 20 aa, Artificial Sequence
  Bos taurus alpha-S1-casein epitope
LNENLLRFFVAPFPQVFGKE

SEQ ID NO: 377 - protein, 10 aa, Artificial Sequence
  Bos taurus Alpha-S1-casein precursor epitope
AMEDIKQMEA

SEQ ID NO: 378 - protein, 10 aa, Artificial Sequence
  Bos taurus Alpha-S2-casein precursor epitope
ENLCSTFCKE

SEQ ID NO: 379 - protein, 15 aa, Artificial Sequence
  Arachis hypogaea Ara h 2.01 allergen epitope
CCNELNEFENNQRCM

SEQ ID NO: 380 - protein, 15 aa, Artificial Sequence
  Glycine max Bd 30K (34 kDa maturing seed protein) epitope
EDWGEDGYIWIQRNT

SEQ ID NO: 381 - protein, 8 aa, Artificial Sequence
  Betula pendula Bet v 4 epitope
FARANRGL

SEQ ID NO: 382 - protein, 9 aa, Artificial Sequence
  Musa acuminata beta-1, 3-glucananse epitope
GLFYPNKQP

SEQ ID NO: 383 - protein, 15 aa, Artificial Sequence
  Hevea brasiliensis beta-1,3-glucanase epitope
GLFFPDKRPKYNLNF

SEQ ID NO: 384 - protein, 12 aa, Artificial Sequence
  Olea europaea beta-1,3-glucanase-like protein epitope
AGRNSWNCDFSQ

SEQ ID NO: 385 - protein, 13 aa, Artificial Sequence
  Bos taurus beta-casein epitope
QSKVLPVPQKAVP

SEQ ID NO: 386 - protein, 12 aa, Artificial Sequence
  Bos taurus Beta-casein precursor epitope
DELQDKIHPFAQ

SEQ ID NO: 387 - protein, 10 aa, Artificial Sequence
  Bos taurus Beta-lactoglobulin epitope
AQKKIIAEKT

SEQ ID NO: 388 - protein, 16 aa, Artificial Sequence
  Bos taurus Beta-lactoglobulin precursor epitope
AASDISLLDAQSAPLR

SEQ ID NO: 389 - protein, 8 aa, Artificial Sequence
  Fagopyrum esculentum BW 16kDa allergen epitope
EGVRDLKE

SEQ ID NO: 390 - protein, 17 aa, Artificial Sequence
  Betula pendula Chain A, Birch Pollen Profilin epitope
AQSSSFPQFKPQEITGI

SEQ ID NO: 391 - protein, 20 aa, Artificial Sequence
  Oncorhynchus mykiss collagen a2(I) epitope
MKGLRGHGGLQGMPGPNGPS

SEQ ID NO: 392 - protein, 46 aa, Artificial Sequence
  Bos taurus collagen, type I, alpha 2 epitope
APGPDGNNGAQGPPGLQGVQGGKGEQGPAGPPGFQGLPGPAGTAGE

SEQ ID NO: 393 - protein, 15 aa, Artificial Sequence
  Arachis hypogaea Conglutin-7 precursor epitope
AAHASARQQWELQGD

SEQ ID NO: 394 - protein, 8 aa, Artificial Sequence
  Periplaneta americana Cr-PII allergen epitope
IRSWFGLP

SEQ ID NO: 395 - protein, 11 aa, Artificial Sequence
  Cochliobolus lunatus Cytochrome c epitope
ENPKKYIPGTK

SEQ ID NO: 396 - protein, 10 aa, Artificial Sequence
  Rattus norvegicus Cytochrome P450 3A1 epitope
DMVLNETLRL

SEQ ID NO: 397 - protein, 9 aa, Artificial Sequence
  Dermatophagoides farinae Der f 2 epitope
IATHAKIRD

SEQ ID NO: 398 - protein, 15 aa, Artificial Sequence
  Dermatophagoides farinae Der f 7 allergen epitope
HIGGLSILDPIFGVL

SEQ ID NO: 399 - protein, 43 aa, Artificial Sequence
  Dermatophagoides pteronyssinus Der p 1 allergen epitope
AREQSCRRPNAQRFGISNYCQIYPPNANKIREALAQTHSAIAV

SEQ ID NO: 400 - protein, 15 aa, Artificial Sequence
  Dermatophagoides pteronyssinus Der p 7 allergen polypeptide epitope
HIGGLSILDPIFAVL

SEQ ID NO: 401 - protein, 39 aa, Artificial Sequence
  Candida albicans Enolase 1 (2-phosphoglycerate dehydratase) (2-phospho-D-glycerate hydro-lyase) epitope
QAANDSYAAGWGVMVSHRSGETEDTFIADLSVGLRSGQI

SEQ ID NO: 402 - protein, 21 aa, Artificial Sequence
  Hevea brasiliensis ENSP-like protein epitope
FPLITCCGYGGKYNFSVTAPC

SEQ ID NO: 403 - protein, 12 aa, Artificial Sequence
  Fagopyrum esculentum Fag e 1 epitope
AVVLKAGNEGLE

SEQ ID NO: 404 - protein, 10 aa, Artificial Sequence
  Triticum aestivum Gamma-gliadin precursor epitope
LQPQQPFPQQ

SEQ ID NO: 405 - protein, 21 aa, Artificial Sequence
  Chironomus thummi thummi Globin CTT-III epitope
AHTDFAGAEAAWGATLDTFFG

SEQ ID NO: 406 - protein, 11 aa, Artificial Sequence
  Chironomus thummi thummi Globin CTT-III precursor epitope
GVTHDQLNNFR

SEQ ID NO: 407 - protein, 23 aa, Artificial Sequence
  Chironomus thummi thummi Globin CTT-IV precursor epitope
KAHTDFAGAEAAWGATLDAFFGM

SEQ ID NO: 408 - protein, 35 aa, Artificial Sequence
  Chironomus thummi thummi Globin CTT-VI precursor epitope
IVSFLSEVISLAGSDANIPAIQNLAKELATSHKPR

SEQ ID NO: 409 - protein, 35 aa, Artificial Sequence
  Chironomus thummi thummi Globin CTT-VIII epitope
IVGFFSEVIGLIGNPENRPALKTLIDGLASSHKAR

SEQ ID NO: 410 - protein, 9 aa, Artificial Sequence
  Hevea brasiliensis Glucan endo-1,3-beta-glucosidase, basic vacuolar isoform epitope
AWLAQFVLP

SEQ ID NO: 411 - protein, 14 aa, Artificial Sequence
  Triticum aestivum Glutenin, high molecular weight subunit DX5 epitope
AQGQQPGQGQQGQQ

SEQ ID NO: 412 - protein, 5 aa, Artificial Sequence
  Triticum aestivum Glutenin, high molecular weight subunit DX5 precursor epitope
QQPGQ

SEQ ID NO: 413 - protein, 5 aa, Artificial Sequence
  Triticum aestivum Glutenin, low molecular weight subunit precursor epitope
QQQPP

SEQ ID NO: 414 - protein, 15 aa, Artificial Sequence
  Phaseolus vulgaris Glycine-rich cell wall structural protein 1.8 precursor epitope
GGYGDGGAHGGGYGG

SEQ ID NO: 415 - protein, 15 aa, Artificial Sequence
  Arachis hypogaea Glycinin epitope
ALSRLVLRRNALRRP

SEQ ID NO: 416 - protein, 13 aa, Artificial Sequence
  Glycine max Glycinin G1 precursor epitope
GAIVTVKGGLSVI

SEQ ID NO: 417 - protein, 15 aa, Artificial Sequence
  Glycine max Glycinin G2 precursor epitope
ALSRCTLNRNALRRP

SEQ ID NO: 418 - protein, 15 aa, Artificial Sequence
  Holcus lanatus group V allergen epitope
ANVPPADKYKTFEAA

SEQ ID NO: 419 - protein, 12 aa, Artificial Sequence
  Oryza sativa Japonica Group hypothetical protein epitope
AFNHFGIQLVQR

SEQ ID NO: 420 - protein, 14 aa, Artificial Sequence
  Bos taurus Kappa-casein precursor epitope
AKYIPIQYVLSRYP

SEQ ID NO: 421 - protein, 20 aa, Artificial Sequence
  Alternaria alternata Major allergen Alt a 1 precursor epitope
ADPVTTEGDYVVKISEFYGR

SEQ ID NO: 422 - protein, 15 aa, Artificial Sequence
  Anisakis simplex Major allergen Ani s 1 epitope
CKMPDRGACALGKKP

SEQ ID NO: 423 - protein, 13 aa, Artificial Sequence
  Aspergillus fumigatus Major allergen Asp f 1 epitope
LNPKTNKWEDKRY

SEQ ID NO: 424 - protein, 10 aa, Artificial Sequence
  Aspergillus fumigatus Major allergen Asp f 2 epitope
AHILRWGNES

SEQ ID NO: 425 - protein, 20 aa, Artificial Sequence
  Bos taurus major allergen beta-lactoglobulin epitope
LQKWENDECAQKKIIAEKTK

SEQ ID NO: 426 - protein, 14 aa, Artificial Sequence
  Felis catus Major allergen I polypeptide chain 1 precursor epitope
DAKMTEEDKENALS

SEQ ID NO: 427 - protein, 14 aa, Artificial Sequence
  Felis catus Major allergen I polypeptide chain 2 precursor epitope
EPERTAMKKIQDCY

SEQ ID NO: 428 - protein, 11 aa, Artificial Sequence
  Felis catus major allergen I, polypeptide chain 1 epitope
LLDKIYTSPLC

SEQ ID NO: 429 - protein, 29 aa, Artificial Sequence
  Turbo cornutus major allergen Tur c1 - Turbo cornutus epitope
LEDELLAEKEKYKAISDELDQTFAELAGY

SEQ ID NO: 430 - protein, 25 aa, Artificial Sequence
  Dermatophagoides pteronyssinus major house dust allergen epitope
LAHRNQSLDLAEQELVDCASQHGCH

SEQ ID NO: 431 - protein, 9 aa, Artificial Sequence
  Hevea brasiliensis Major latex allergen Hev b 5 epitope
APPASEQET

SEQ ID NO: 432 - protein, 43 aa, Artificial Sequence
  Dermatophagoides pteronyssinus Major mite fecal allergen Der p 1 epitope
AREQSCRRPNAQRFGISNYCQIYPPNANKIREALAQPQRYCRH

SEQ ID NO: 433 - protein, 12 aa, Artificial Sequence
  Olea europaea Major pollen allergen epitope
FTEVGYTRAEGL

SEQ ID NO: 434 - protein, 10 aa, Artificial Sequence
  Betula pendula Major pollen allergen Bet v 1-A epitope
DGDNLFPKVA

SEQ ID NO: 435 - protein, 11 aa, Artificial Sequence
  Chamaecyparis obtusa Major pollen allergen Cha o 1 precursor epitope
WRSTQDSFNNG

SEQ ID NO: 436 - protein, 17 aa, Artificial Sequence
  Corylus avellana Major pollen allergen Cor a 1 epitope
YVLDGDKLLPKVAPQAL

SEQ ID NO: 437 - protein, 27 aa, Artificial Sequence
  Holcus lanatus Major pollen allergen Hol l 1 precursor epitope
AKSTWYGKPTGAGPKDNGGACGYKDVD

SEQ ID NO: 438 - protein, 12 aa, Artificial Sequence
  Juniperus ashei Major pollen allergen Jun a 1 precursor epitope
AFNQFGPNAGQR

SEQ ID NO: 439 - protein, 34 aa, Artificial Sequence
  Olea europaea major pollen allergen Ole e 1 epitope
SGRKDCNEIPTEGWVKPSLKFILNTVNGTTRTVN

SEQ ID NO: 440 - protein, 9 aa, Artificial Sequence
  Malus x domestica mal d 3 epitope
RTTADRQTA

SEQ ID NO: 441 - protein, 16 aa, Artificial Sequence
  Blomia tropicalis Mite allergen Blo t 5 epitope
EEAQTLSKILLKDLKE

SEQ ID NO: 442 - protein, 5 aa, Artificial Sequence
  Dermatophagoides farinae Mite group 2 allergen Der f 2 precursor epitope
DPCII

SEQ ID NO: 443 - protein, 15 aa, Artificial Sequence
  Dermatophagoides pteronyssinus Mite group 2 allergen Der p 2 precursor epitope
DQVDVKDCANHEIKK

SEQ ID NO: 444 - protein, 33 aa, Artificial Sequence
  Lepidoglyphus destructor Mite group 2 allergen Lep d 2 precursor epitope
AANQDTAKVTIKVLAKVAGTTIQVPGLETDGCK

SEQ ID NO: 445 - protein, 6 aa, Artificial Sequence
  Triticum aestivum monomeric alpha-amylase inhibitor epitope
AASVPE

SEQ ID NO: 446 - protein, 9 aa, Artificial Sequence
  Prunus armeniaca Non-specific lipid-transfer protein 1 epitope
VNPNNAAAL

SEQ ID NO: 447 - protein, 15 aa, Artificial Sequence
  Prunus armeniaca Non-specific lipid-transfer protein 1 (LTP 1) (Major allergen Pru ar 3) epitope
LARTTPDRRTACNCL

SEQ ID NO: 448 - protein, 18 aa, Artificial Sequence
  Prunus domestica Non-specific lipid-transfer protein 1 (LTP 1) (Major allergen Pru d 3) epitope
LARTTADRRAACNCLKQL

SEQ ID NO: 449 - protein, 15 aa, Artificial Sequence
  Malus x domestica Non-specific lipid-transfer protein precursor (LTP) (Allergen Mal d 3) epitope
ADRQTACNCLKNLAG

SEQ ID NO: 450 - protein, 12 aa, Artificial Sequence
  Olea europaea Ole e 1 protein epitope
EDVPQPPVSQFH

SEQ ID NO: 451 - protein, 25 aa, Artificial Sequence
  Olea europaea Ole e 1.0102 protein epitope
EDVPQPPVSQFHIQGQVYCDTCRAG

SEQ ID NO: 452 - protein, 10 aa, Artificial Sequence
  Triticum aestivum Omega gliadin storage protein epitope
QQPQQSFPQQ

SEQ ID NO: 453 - protein, 7 aa, Artificial Sequence
  Triticum aestivum omega-5 gliadin epitope
QQFHQQQ

SEQ ID NO: 454 - protein, 35 aa, Artificial Sequence
  Aspergillus fumigatus Oryzin precursor epitope
ASNTSPASAPNALTVAAINKSNARASFSNYGSVVD

SEQ ID NO: 455 - protein, 9 aa, Artificial Sequence
  Gallus gallus Ovalbumin epitope
CFDVFKELK

SEQ ID NO: 456 - protein, 10 aa, Artificial Sequence
  Gallus gallus Ovomucoid epitope
CNFCNAVVES

SEQ ID NO: 457 - protein, 14 aa, Artificial Sequence
  Gallus gallus Ovomucoid precursor epitope
AEVDCSRFPNATDK

SEQ ID NO: 458 - protein, 10 aa, Artificial Sequence
  Glycine max P34 probable thiol protease precursor epitope
ASWDWRKKGV

SEQ ID NO: 459 - protein, 10 aa, Artificial Sequence
  Glycine max P34 probable thiol protease precursor; Gly m 1 epitope
PQEFSKKTYQ

SEQ ID NO: 460 - protein, 9 aa, Artificial Sequence
  Parietaria judaica Par j epitope
GTSSCRLVP

SEQ ID NO: 461 - protein, 47 aa, Artificial Sequence
  Blomia tropicalis Paramyosin epitope
EKLRDQKEALARENKKLADDLAEAKSQLNDAHRRIHEQEIEIKRLEN

SEQ ID NO: 462 - protein, 8 aa, Artificial Sequence
  Gadus morhua callarias Parvalbumin beta epitope
AAEAACFK

SEQ ID NO: 463 - protein, 15 aa, Artificial Sequence
  Salmo salar parvalbumin like 1 epitope
ADIKTALEARKAADT

SEQ ID NO: 464 - protein, 12 aa, Artificial Sequence
  Juniperus ashei Pathogenesis-related protein precursor epitope
ADINAVCPSELK

SEQ ID NO: 465 - protein, 12 aa, Artificial Sequence
  Nicotiana tabacum Pectate lyase epitope
AYNHFGKRLDQR

SEQ ID NO: 466 - protein, 12 aa, Artificial Sequence
  Musa acuminata AAA Group pectate lyase 2 epitope
AFNHFGEGLIQR

SEQ ID NO: 467 - protein, 15 aa, Artificial Sequence
  Farfantepenaeus aztecus Pen a 1 allergen epitope
ANIQLVEKDKALSNA

SEQ ID NO: 468 - protein, 43 aa, Artificial Sequence
  Dermatophagoides pteronyssinus Peptidase 1 precursor (Major mite fecal allergen Der p 1) (Allergen Der p I) epitope
AREQSCRRPNAQRFGISNYCQIYPPNVNKIREALAQTHSAIAV

SEQ ID NO: 469 - protein, 45 aa, Artificial Sequence
  Apis mellifera Phospholipase A2 precursor epitope
LIDTKCYKLEHPVTGCGERTEGRCLHYTVDKSKPKVYQWFDLRKY

SEQ ID NO: 470 - protein, 14 aa, Artificial Sequence
  Myrmecia pilosula Pilosulin-1 precursor (Major allergen Myr p 1) (Myr p I) epitope
KEAIPMAVEMAKSQ

SEQ ID NO: 471 - protein, 8 aa, Artificial Sequence
  Betula pendula Polcalcin Bet v 4 epitope
FGRANRGL

SEQ ID NO: 472 - protein, 36 aa, Artificial Sequence
  Phleum pratense Polcalcin Phl p 7 (Calcium-binding pollen allergen Phl p 7) (P7) epitope
ADDMERIFKRFDTNGDGKISLSELTDALRTLGSTSA

SEQ ID NO: 473 - protein, 25 aa, Artificial Sequence
  Lolium perenne pollen allergen epitope
EGGTKSEVEDVIPEGWKADTSYSAK

SEQ ID NO: 474 - protein, 12 aa, Artificial Sequence
  Ambrosia artemisiifolia Pollen allergen Amb a 1.4 epitope
AFNKFTDNVDQR

SEQ ID NO: 475 - protein, 8 aa, Artificial Sequence
  Ambrosia artemisiifolia Pollen allergen Amb a 2 precursor epitope
MPRCRFGF

SEQ ID NO: 476 - protein, 15 aa, Artificial Sequence
  Ambrosia artemisiifolia var. elatior Pollen allergen Amb a 3 epitope
CDIKDPIRLEPGGPD

SEQ ID NO: 477 - protein, 31 aa, Artificial Sequence
  Betula pendula pollen allergen Bet v 1 epitope
KAEQVKASKEMGETLLRAVESYLLAHSDAYN

SEQ ID NO: 478 - protein, 20 aa, Artificial Sequence
  Poa pratensis Pollen allergen KBG 60 precursor epitope
AANKYKTFVATFGAASNKAF

SEQ ID NO: 479 - protein, 25 aa, Artificial Sequence
  Lolium perenne Pollen allergen Lol p 2-A (Lol p II-A) epitope
EKGMRNVFDDVVPADFKVGTTYKPE

SEQ ID NO: 480 - protein, 27 aa, Artificial Sequence
  Lolium perenne Pollen allergen Lol p 3 (Lol p III) epitope
KGGMKNVFDEVIPTAFTVGKTYTPEYN

SEQ ID NO: 481 - protein, 12 aa, Artificial Sequence
  Lolium perenne Pollen allergen Lol p VA precursor epitope
AAEGATPEAKYD

SEQ ID NO: 482 - protein, 15 aa, Artificial Sequence
  Phleum pratense Pollen allergen Phl p 1 precursor epitope
APYHFDLSGHAFGAM

SEQ ID NO: 483 - protein, 8 aa, Artificial Sequence
  Zea mays pollen allergen Phl p 11 epitope
RDRARVPL

SEQ ID NO: 484 - protein, 12 aa, Artificial Sequence
  Phleum pratense pollen allergen Phl pI epitope
IPKVPPGPNITA

SEQ ID NO: 485 - protein, 20 aa, Artificial Sequence
  Cryptomeria japonica Polygalacturonase precursor epitope
GQCKWVNGREICNDRDRPTA

SEQ ID NO: 486 - protein, 30 aa, Artificial Sequence
  Parietaria judaica Probable non-specific lipid-transfer protein epitope
QETCGTMVRALMPCLPFVQGKEKEPSKGCC

SEQ ID NO: 487 - protein, 10 aa, Artificial Sequence
  Parietaria judaica Probable non-specific lipid-transfer protein 2 epitope
AEVPKKCDIK

SEQ ID NO: 488 - protein, 30 aa, Artificial Sequence
  Parietaria judaica Probable non-specific lipid-transfer protein 2 precursor epitope
EACGKVVQDIMPCLHFVKGEEKEPSKECCS

SEQ ID NO: 489 - protein, 12 aa, Artificial Sequence
  Solanum lycopersicum Probable pectate lyase P59 epitope
AFNHFGKRLIQR

SEQ ID NO: 490 - protein, 10 aa, Artificial Sequence
  Cucumis melo profilin epitope
AFRLEEIAAI

SEQ ID NO: 491 - protein, 56 aa, Artificial Sequence
  Glycine max Profilin-1 epitope
WAQSTDFPQFKPEEITAIMNDFNEPGSLAPTGLYLGGTKYMVIQGEPGAVIRGKKG

SEQ ID NO: 492 - protein, 43 aa, Artificial Sequence; identical to SEQ ID NO: 292
  Hevea brasiliensis Pro-hevein precursor epitope

SEQ ID NO: 493 - protein, 10 aa, Artificial Sequence
  Prunus persica pru p 1 epitope
GKCGVSIPYK

SEQ ID NO: 494 - protein, 15 aa, Artificial Sequence
  Prunus dulcis prunin 1 precursor epitope
EESQQSSQQGRQQEQ

SEQ ID NO: 495 - protein, 15 aa, Artificial Sequence
  Prunus dulcis prunin 2 precursor epitope
DSQPQQFQQQQQQQQ

SEQ ID NO: 496 - protein, 11 aa, Artificial Sequence
  Hesperocyparis arizonica putative allergen Cup a 1 epitope
WRFTRDAFTNG

SEQ ID NO: 497 - protein, 10 aa, Artificial Sequence
  Aspergillus fumigatus Ribonuclease mitogillin precursor epitope
FPTFPDGHDY

SEQ ID NO: 498 - protein, 12 aa, Artificial Sequence
  Mangifera indica ripening-related pectate lyase epitope
AYNHFGEGLIQR

SEQ ID NO: 499 - protein, 10 aa, Artificial Sequence
  Hevea brasiliensis Rubber elongation factor protein epitope
AEDEDNQQGQ

SEQ ID NO: 500 - protein, 15 aa, Artificial Sequence
  Juglans regia seed storage protein epitope
DDNGLEETICTLRLR

SEQ ID NO: 501 - protein, 15 aa, Artificial Sequence
  Arachis hypogaea seed storage protein SSP2 epitope
CGLRAPQRCDLDVES

SEQ ID NO: 502 - protein, 8 aa, Artificial Sequence
  Gallus gallus serine (or cysteine) proteinase inhibitor, clade B (ovalbumin), member 3 epitope
RPNATYSL

SEQ ID NO: 503 - protein, 8 aa, Artificial Sequence
  Gallus gallus Serum albumin epitope
QSRATLGI

SEQ ID NO: 504 - protein, 17 aa, Artificial Sequence
  Bos taurus Serum albumin precursor epitope
DDSPDLPKLKPDPNTLC

SEQ ID NO: 505 - protein, 10 aa, Artificial Sequence
  Hevea brasiliensis Small rubber particle protein epitope
AEEVEEERLK

SEQ ID NO: 506 - protein, 12 aa, Artificial Sequence
  Cryptomeria japonica Sugi basic protein precursor epitope
DALTLRTATNIW

SEQ ID NO: 507 - protein, 48 aa, Artificial Sequence
  Aspergillus fumigatus Superoxide dismutase epitope
YTLPPLPYPYDALQPYISQQIMELHHKKHHQTYVNGLNAALEAQKKAA

SEQ ID NO: 508 - protein, 20 aa, Artificial Sequence
  Trichophyton rubrum Tri r 2 allergen epitope
DCNGHGTHVAGTVGGTKYGL

SEQ ID NO: 509 - protein, 10 aa, Artificial Sequence
  Triticum aestivum Triticum aestivum proteins epitope
LPQQQIPQQP

SEQ ID NO: 510 - protein, 9 aa, Artificial Sequence
  Penaeus tropomyosin epitope
FLAEEADRK

SEQ ID NO: 511 - protein, 20 aa, Artificial Sequence
  Paralichthys olivaceus type 1 collagen alpha 2 epitope
MKGLRGHPGLQGMPGPSGPS

SEQ ID NO: 512 - protein, 10 aa, Artificial Sequence
  Triticum aestivum type 1 non-specific lipid transfer protein precursor epitope
ARGTPLKCGV

SEQ ID NO: 513 - protein, 18 aa, Artificial Sequence
  Anisakis simplex UA3-recognized allergen epitope
MCQCVQKYGTEFCKKRLA

SEQ ID NO: 514 - protein, 8 aa, Artificial Sequence
  Juglans nigra vicilin seed storage protein epitope
SFEDQGRR

SEQ ID NO: 515 - protein, 15 aa, Artificial Sequence
  Anacardium occidentale Vicilin-like protein epitope
AIMGPPTKFSFSLFL

SEQ ID NO: 516 - protein, 10 aa, Artificial Sequence
  Juglans regia vicilin-like protein precursor epitope
DQRSQEERER